European Patent Specification EP 3 362 472 B1, published August 30, 2023. Title: COMPOSITIONS AND METHODS FOR INHIBITION OF LINEAGE SPECIFIC ANTIGENS. Applicant: The Trustees of Columbia University in the City of New York. Application Not Yet Assigned. The sequence listing filed with the application follows.

SEQUENCE LISTING (47 sequences)

SEQ ID NO: 1 - DNA, 339 bp, Homo sapiens
gagatcgtgctgacccagagccccggcagcctggccgtgagccccggcgagagggtgaccatgagctgcaagagcagccagagcgtgttcttcagcagcagccagaagaactacctggcctggtaccagcagatccccggccagagccccaggctgctgatctactgggccagcaccagggagagcggcgtgcccgacaggttcaccggcagcggcagcggcaccgacttcaccctgaccatcagcagcgtgcagcccgaggacctggccatctactactgccaccagtacctgagcagcaggaccttcggccagggcaccaagctggagatcaagagg

SEQ ID NO: 2 - DNA, 354 bp, Homo sapiens
caggtgcagctgcagcagcccggcgccgaggtggtgaagcccggcgccagcgtgaagatgagctgcaaggccagcggctacaccttcaccagctactacatccactggatcaagcagacccccggccagggcctggagtgggtgggcgtgatctaccccggcaacgacgacatcagctacaaccagaagttccagggcaaggccaccctgaccgccgacaagagcagcaccaccgcctacatgcagctgagcagcctgaccagcgaggacagcgccgtgtactactgcgccagggaggtgaggctgaggtacttcgacgtgtggggccagggcaccaccgtgaccgtgagcagc

SEQ ID NO: 3 - DNA, 657 bp, Homo sapiens
attgaagttatgtatcctcctccttacctagacaatgagaagagcaatggaaccattatccatgtgaaagggaaacacctttgtccaagtcccctatttcccggaccttctaagcccttttgggtgctggtggtggttggtggagtcctggcttgctatagcttgctagtaacagtggcctttattattttctgggtgaggagtaagaggagcaggctcctgcacagtgactacatgaacatgactccccgccgccccgggcccacccgcaagcattaccagccctatgccccaccacgcgacttcgcagcctatcgctccagagtgaagttcagcaggagcgcagacgcccccgcgtaccagcagggccagaaccagctctataacgagctcaatctaggacgaagagaggagtacgatgttttggacaagagacgtggccgggaccctgagatggggggaaagccgagaaggaagaaccctcaggaaggcctgtacaatgaactgcagaaagataagatggcggaggcctacagtgagattgggatgaaaggcgagcgccggaggggcaaggggcacgatggcctttaccagggtctcagtacagccaccaaggacacctacgacgcccttcacatgcaggccctgccccctcgc

SEQ ID NO: 4 - DNA, 603 bp, Homo sapiens
ctatcaatttttgatcctcctccttttaaagtaactcttacaggaggatatttgcatatttatgaatcacaactttgttgccagctgaagttctggttacccataggatgtgcagcctttgttgtagtctgcattttgggatgcatacttatttgttggcttacaaaaaagaagtattcatccagtgtgcacgaccctaacggtgaatacatgttcatgagagcagtgaacacagccaaaaaatctagactcacagatgtgaccctaagagtgaagttcagcaggagcgcagacgcccccgcgtaccagcagggccagaaccagctctataacgagctcaatctaggacgaagagaggagtacgatgttttggacaagagacgtggccgggaccctgagatggggggaaagccgagaaggaagaaccctcaggaaggcctgtacaatgaactgcagaaagataagatggcggaggcctacagtgagattgggatgaaaggcgagcgccggaggggcaaggggcacgatggcctttaccagggtctcagtacagccaccaaggacacctacgacgcccttcacatgcaggccctgccccctcgc

SEQ ID NO: 5 - DNA, 627 bp, Homo sapiens
attgaagttatgtatcctcctccttacctagacaatgagaagagcaatggaaccattatccatgtgaaagggaaacacctttgtccaagtcccctatttcccggaccttctaagcccttttgggtgctggtggtggttggtggagtcctggcttgctatagcttgctagtaacagtggcctttattattttctgggtgaggagtaagaggagcaggctcctgcacagtgactacatgttcatgagagcagtgaacacagccaaaaaatctagactcacagatgtgaccctaagagtgaagttcagcaggagcgcagacgcccccgcgtaccagcagggccagaaccagctctataacgagctcaatctaggacgaagagaggagtacgatgttttggacaagagacgtggccgggaccctgagatggggggaaagccgagaaggaagaaccctcaggaaggcctgtacaatgaactgcagaaagataagatggcggaggcctacagtgagattgggatgaaaggcgagcgccggaggggcaaggggcacgatggcctttaccagggtctcagtacagccaccaaggacacctacgacgcccttcacatgcaggccctgccccctcgc

SEQ ID NO: 6 - protein, 107 aa, Artificial Sequence
  Synthetic Polypeptide
IEVMYPPPYLDNEKSNGTIIHVKGKHLCPSPLFPGPSKPFWVLVVVGGVLACYSLLVTVAFIIFWVRSKRSRLLHSDYMNMTPRRPGPTRKHYQPYAPPRDFAAYRS

SEQ ID NO: 7 - protein, 89 aa, Artificial Sequence
  Synthetic Polypeptide
LSIFDPPPFKVTLTGGYLHIYESQLCCQLKFWLPIGCAAFVVVCILGCILICWLTKKKYSSSVHDPNGEYMFMRAVNTAKKSRLTDVTL

SEQ ID NO: 8 - protein, 97 aa, Artificial Sequence
  Synthetic Polypeptide
IEVMYPPPYLDNEKSNGTIIHVKGKHLCPSPLFPGPSKPFWVLVVVGGVLACYSLLVTVAFIIFWVRSKRSRLLHSDYMFMRAVNTAKKSRLTDVTL

SEQ ID NO: 9 - DNA, 23 bp, Artificial Sequence
  Synthetic Polynucleotide
ccaaagagtccggggatacttgg

SEQ ID NO: 10 - DNA, 23 bp, Artificial Sequence
  Synthetic Polynucleotide
gttgagttttgcattggcggcgg

SEQ ID NO: 11 - DNA, 23 bp, Artificial Sequence
  Synthetic Polynucleotide
acctgtcaggtgaagttcgctgg

SEQ ID NO: 12 - protein, 118 aa, Homo sapiens
QVQLQQPGAEVVKPGASVKMSCKASGYTFTSYYIHWIKQTPGQGLEWVGVIYPGNDDISYNQKFQGKATLTADKSSTTAYMQLSSLTSEDSAVYYCAREVRLRYFDVWGQGTTVTVSS

SEQ ID NO: 13 - protein, 113 aa, Homo sapiens
EIVLTQSPGSLAVSPGERVTMSCKSSQSVFFSSSQKNYLAWYQQIPGQSPRLLIYWASTRESGVPDRFTGSGSGTDFTLTISSVQPEDLAIYYCHQYLSSRTFGQGTKLEIKR

SEQ ID NO: 14 - protein, 19 aa, Artificial Sequence
  Synthetic Polypeptide
GSTSSGSGKPGSGEGSTKG

SEQ ID NO: 15 - protein, 113 aa, Artificial Sequence
  Synthetic Polypeptide
RVKFSRSADAPAYQQGQNQLYNELNLGRREEYDVLDKRRGRDPEMGGKPQRRKNPQEGLYNELQKDKMAEAYSEIGMKGERRRGKGHDGLYQGLSTATKDTYDALHMQALPPR

SEQ ID NO: 16 - DNA, 850 bp, Artificial Sequence
  Synthetic Polynucleotide
ggtgtcgtgagcggccgctgaactggccaccatggacatgagggtccctgctcagctcctggggctcctgctgctctggctctcaggtgccagatgtgagatcgtgctgacccagagccccggcagcctggccgtgagccccggcaagagggtgaccatgagctgcaagagcagccagagcgtgttcttcagcagcagccagaagaactacctggcctggtaccagcagatccccggccagagccccaggctgctgatctactgggccagcaccagggagagcggcgtgcccgacaggttcaccggcagcggcagcggcagcggcaccgacttcaccctgaccatcagcagcgtgcagcccgaggacctggccatctactactgccaccagtacctgagcagcaggaccttcggccagggcaccaagctggagatcaagaggggcagcaccagcggcagcggcaagcccggcagcggcgagggcagcaccaagggccaggtgcagctgcagcagcccggcgccgaggtggtgaagcccggcgccagcgtgaagatgagctgcaaggccagcggctacaccttcaccagctactacatccactggatcaagcagacccccggccagggcctggagtgggtgggcgtgatctaccccggcaacgacgacatcagctacaaccagaagttccagggcaaggccaccctgaccgccgacaagagcagcaccaccgcctacatgcagctgagcagcctgaccagcgaggacagcgccgtgtactactgcgccagggaggtgaggctgaggtacttcgacgtgtggggccagggcaccaccgtgaccgtgagcagc

SEQ ID NO: 17 - DNA, 695 bp, Artificial Sequence
  Synthetic Polynucleotide
gcggccgcaattgaagttatgtatcctcctccttacctagacaatgagaagagcaatggaaccattatccatgtgaaagggaaacacctttgtccaagtcccctatttcccggaccttctaagcccttttgggtgctggtggtggttggtggagtcctggcttgctatagcttgctagtaacagtggcctttattattttctgggtgaggagtaagaggagcaggctcctgcacagtgactacatgaacatgactccccgccgccccgggcccacccgcaagcattaccagccctatgccccaccacgcgacttcgcagcctatcgctccagagtgaagttcagcaggagcgcagacgcccccgcgtaccagcagggccagaaccagctctataacgagctcaatctaggacgaagagaggagtacgatgttttggacaagagacgtggccgggaccctgagatggggggaaagccgagaaggaagaaccctcaggaaggcctgtacaatgaactgcagaaagataagatggcggaggcctacagtgagattgggatgaaaggcgagcgccggaggggcaaggggcacgatggcctttaccagggtctcagtacagccaccaaggacacctacgacgcccttcacatgcaggccctgccccctcgctaacgcccctctccctcccccccccctaa

SEQ ID NO: 18 - DNA, 641 bp, Artificial Sequence
  Synthetic Polynucleotide
gcggccgcactatcaatttttgatcctcctccttttaaagtaactcttacaggaggatatttgcatatttatgaatcacaactttgttgccagctgaagttctggttacccataggatgtgcagcctttgttgtagtctgcattttgggatgcatacttatttgttggcttacaaaaaagaagtattcatccagtgtgcacgaccctaacggtgaatacatgttcatgagagcagtgaacacagccaaaaaatctagactcacagatgtgaccctaagagtgaagttcagcaggagcgcagacgcccccgcgtaccagcagggccagaaccagctctataacgagctcaatctaggacgaagagaggagtacgatgttttggacaagagacgtggccgggaccctgagatggggggaaagccgagaaggaagaaccctcaggaaggcctgtacaatgaactgcagaaagataagatggcggaggcctacagtgagattgggatgaaaggcgagcgccggaggggcaaggggcacgatggcctttaccagggtctcagtacagccaccaaggacacctacgacgcccttcacatgcaggccctgccccctcgctaacgcccctctccctcccccccccctaa

SEQ ID NO: 19 - DNA, 665 bp, Artificial Sequence
  Synthetic Polynucleotide
gcggccgcaattgaagttatgtatcctcctccttacctagacaatgagaagagcaatggaaccattatccatgtgaaagggaaacacctttgtccaagtcccctatttcccggaccttctaagcccttttgggtgctggtggtggttggtggagtcctggcttgctatagcttgctagtaacagtggcctttattattttctgggtgaggagtaagaggagcaggctcctgcacagtgactacatgttcatgagagcagtgaacacagccaaaaaatctagactcacagatgtgaccctaagagtgaagttcagcaggagcgcagacgcccccgcgtaccagcagggccagaaccagctctataacgagctcaatctaggacgaagagaggagtacgatgttttggacaagagacgtggccgggaccctgagatggggggaaagccgagaaggaagaaccctcaggaaggcctgtacaatgaactgcagaaagataagatggcggaggcctacagtgagattgggatgaaaggcgagcgccggaggggcaaggggcacgatggcctttaccagggtctcagtacagccaccaaggacacctacgacgcccttcacatgcaggccctgccccctcgctaacgcccctctccctcccccccccctaa

SEQ ID NO: 20 - protein, 503 aa, Homo sapiens
MWLQSLLLLGTVACSISEIVLTQSPGSLAVSPGERVTMSCKSSQSVFFSSSQKNYLAWYQQIPGQSPRLLIYWASTRESGVPDRFTGSGSGTDFTLTISSVQPEDLAIYYCHQYLSSRTFGQGTKLEIKRGSTSGSGKPGSGEGSTKGQVQLQQPGAEVVKPGASVKMSCKASGYTFTSYYIHWIKQTPGQGLEWVGVIYPGNDDISYNQKFQGKATLTADKSSTTAYMQLSSLTSEDSAVYYCAREVRLRYFDVWGQGTTVTVSSALSNSIMYFSHFVPVFLPAKPTTTPAPRPPTPAPTIASQPLSLRPEASRPAAGGAVHTRGLDIYIWAPLAGTCGVLLLSLVITKRGRKKLLYIFKQPFMRPVQTTQEEDGCSCRFPEEEEGGCELRVKFSRSADAPAYQQGQNQLYNELNLGRREEYDVLDKRRGRDPEMGGKPRRKNPQEGLYNELQKDKMAEAYSEIGMKGERRRGKGHDGLYQGLSTATKDTYDALHMQALPPR

SEQ ID NO: 21 - protein, 509 aa, Homo sapiens
MWLQSLLLLGTVACSISEIVLTQSPGSLAVSPGERVTMSCKSSQSVFFSSSQKNYLAWYQQIPGQSPRLLIYWASTRESGVPDRFTGSGSGTDFTLTISSVQPEDLAIYYCHQYLSSRTFGQGTKLEIKRGSTSGSGKPGSGEGSTKGQVQLQQPGAEVVKPGASVKMSCKASGYTFTSYYIHWIKQTPGQGLEWVGVIYPGNDDISYNQKFQGKATLTADKSSTTAYMQLSSLTSEDSAVYYCAREVRLRYFDVWGQGTTVTVSALSNSIMYFSHFVPVFLPAKPTTTPAPRPPTPAPTIASQPLSLRPEASRPAAGGAVHTRGLDKPFWVLVVVGGVLACYSLLVTVAFIIFWVRSKRSRLLHSDYMNMTPRRPGPTRKHYQPYAPPRDFAAYRSRVKFSRSADAPAYQQGQNQLYNELNLGRREEYDVLDKRRGRDPEMGGKPRRKNPQEGLYNELQKDKMAEAYSEIGMKGERRRGKGHDGLYQGLSTATKDTYDALHMQALPPR

SEQ ID NO: 22 - protein, 552 aa, Homo sapiens
MWLQSLLLLGTVACSISEIVLTQSPGSLAVSPGERVTMSCKSSQSVFFSSSQKNYLAWYQQIPGQSPRLLIYWASTRESGVPDRFTGSGSGTDFTLTISSVQPEDLAIYYCHQYLSSRTFGQGTKLEIKRGSTSGSGKPGSGEGSTKGQVQLQQPGAEVVKPGASVKMSCKASGYTFTSYYIHWIKQTPGQGLEWVGVIYPGNDDISYNQKFQGKATLTADKSSTTAYMQLSSLTSEDSAVYYCAREVRLRYFDVWGQGTTVTVSSALSNSIMYFSHFVPVFLPAKPTTTPAPRPPTPAPTIASQPLSLRPEASRPAAGGAVHTRGLDKPFWVLVVVGGVLACYSLLVTVAFIIFWVRSKRSRLLHSDYMNMTPRRPGPTRKHYQPYAPPRDFAAYRSKRGRKKLLYIFKQPFMRPVQTTQEEDGCSCRFPEEEEGGCELRVKFSRSADAPAYQQGQNQLYNELNLGRREEYDVLDKRRGRDPEMGGKPRRKNPQEGLYNELQKDKMAEAYSEIGMKGERRRGKGHDGLYQGLSTATKDTYDALHMQALPPR

SEQ ID NO: 23 - protein, 542 aa, Homo sapiens
MWLQSLLLLGTVACSISEIVLTQSPGSLAVSPGERVTMSCKSSQSVFFSSSQKNYLAWYQQIPGQSPRLLIYWASTRESGVPDRFTGSGSGTDFTLTISSVQPEDLAIYYCHQYLSSRTFGQGTKLEIKRGSTSGSGKPGSGEGSTKGQVQLQQPGAEVVKPGASVKMSCKASGYTFTSYYIHWIKQTPGQGLEWVGVIYPGNDDISYNQKFQGKATLTADKSSTTAYMQLSSLTSEDSAVYYCAREVRLRYFDVWGQGTTVTVSSALSNSIMYFSHFVPVFLPAKPTTTPAPRPPTPAPTIASQPLSLRPEASRPAAGGAVHTRGLDFWLPIGCAAFVVVCILGCILICWLTKKKYSSSVHDPNGEYMFMRAVNTAKKSRLTDVTLTKRGRKKLLYIFKQPFMRPVQTTQEEDGCSCRFPEEEEGGCELRVKFSRSADAPAYQQGQNQLYNELNLGRREEYDVLDKRRGRDPEMGGKPRRKNPQEGLYNELQKDKMAEAYSEIGMKGERRRGKGHDGLYQGLSTATKDTYDALHMQALPPR

SEQ ID NO: 24 - protein, 459 aa, Homo sapiens
MWLQSLLLLGTVACSISIQMTQTTSSLSASLGDRVTISCRASQDISKYLNWYQQKPDGTVKLLIYHTSRLHSGVPSRFSGSGSGTDYSLTISNLEQEDIATYFCQQGNTLPYTFGGGTKLEIGSTSGSGKPGSGEGSTKGLQESGPGLVAPSQSLSVTCTVSGVSLPDYGVSWIRQPPRKGLEWLGVIWGSETTYYNSALKSRLTIIKDNSKSQVFLKMNSLQTDDTAIYYCAKHYYYGGSYAMDYWGQGTSVTVSALSNSIMYFSHFVPVFLPAKPTTTPAPRPPTPAPTIASQPLSLRPEASRPAAGGAVHTRGLDKPFWVLVVVGGVLACYSLLVTVAFIIFWVRVKFSRSADAPAYQQGQNQLYNELNLGRREEYDVLDKRRGRDPEMGGKPRRKNPQEGLYNELQKDKMAEAYSEIGMKGERRRGKGHDGLYQGLSTATKDTYDALHMQALPPR

SEQ ID NO: 25 - protein, 398 aa, Homo sapiens
MWLQSLLLLGTVACSISEIVLTQSPGSLAVSPGERVTMSCKSSQSVFFSSSQKNYLAWYQQIPGQSPRLLIYWASTRESGVPDRFTGSGSGTDFTLTISSVQPEDLAIYYCHQYLSSRTFGQGTKLEIKRGSTSGSGKPGSGEGSTKGQVQLQQPGAEVVKPGASVKMSCKASGYTFTSYYIHWIKQTPGQGLEWVGVIYPGNDDISYNQKFQGKATLTADKSSTTAYMQLSSLTSEDSAVYYCAREVRLRYFDVWGQGTTVTVSSALSNSIMYFSHFVPVFLPAKPTTTPAPRPPTPAPTIASQPLSLRPEASRPAAGGAVHTRGLDKPFWVLVVVGGVLACYSLLVTVAFIIFWVRSKRSRLLHSDYMNMTPRRPGPTRKHYQPYAPPRDFAAYRS

SEQ ID NO: 26 - protein, 500 aa, Homo sapiens
MWLQSLLLLGTVACSISIQMTQTTSSLSASLGDRVTISCRASQDISKYLNWYQQKPDGTVKLLIYHTSRLHSGVPSRFSGSGSGTDYSLTISNLEQEDIATYFCQQGNTLPYTFGGGTKLEIGSTSGSGKPGSGEGSTKGLQESGPGLVAPSQSLSVTCTVSGVSLPDYGVSWIRQPPRKGLEWLGVIWGSETTYYNSALKSRLTIIKDNSKSQVFLKMNSLQTDDTAIYYCAKHYYYGGSYAMDYWGQGTSVTVSALSNSIMYFSHFVPVFLPAKPTTTPAPRPPTPAPTIASQPLSLRPEASRPAAGGAVHTRGLDKPFWVLVVVGGVLACYSLLVTVAFIIFWVRSKRSRLLHSDYMNMTPRRPGPTRKHYQPYAPPRDFAAYRSRVKFSRSADAPAYQQGQNQLYNELNLGRREEYDVLDKRRGRDPEMGGKPRRKNPQEGLYNELQKDKMAEAYSEIGMKGERRRGKGHDGLYQGLSTATKDTYDALHMQALPPR

SEQ ID NO: 27 - protein, 484 aa, Homo sapiens
MWLQSLLLLGTVACSISEIVLTQSPGSLAVSPGERVTMSCKSSQSVFFSSSQKNYLAWYQQIPGQSPRLLIYWASTRESGVPDRFTGSGSGTDFTLTISSVQPEDLAIYYCHQYLSSRTFGQGTKLEIKRGSTSGSGKPGSGEGSTKGQVQLQQPGAEVVKPGASVKMSCKASGYTFTSYYIHWIKQTPGQGLEWVGVIYPGNDDISYNQKFQGKATLTADKSSTTAYMQLSSLTSEDSAVYYCAREVRLRYFDVWGQGTTVTVSSIEVMYPPPYLDNEKSNGTIIHVKGKHLCPSPLFPGPSKPFWVLVVVGGVLACYSLLVTVAFIIFWVRSKRSRLLHSDYMNMTPRRPGPTRKHYQPYAPPRDFAAYRSRVKFSRSADAPAYQQGQNQLYNELNLGRREEYDVLDKRRGRDPEMGGKPRRKNPQEGLYNELQKDKMAEAYSEIGMGERRRGKGHDGLYQGLSTATKDTYDALHMQALPPR

SEQ ID NO: 28 - DNA, 23 bp, Artificial Sequence
  Synthetic Polynucleotide
tggccgggttctagagtgccagg

SEQ ID NO: 29 - DNA, 23 bp, Artificial Sequence
  Synthetic Polynucleotide
ggccgggttctagagtgccaggg

SEQ ID NO: 30 - DNA, 23 bp, Artificial Sequence
  Synthetic Polynucleotide
caccgaggagtgagtagtcctgg

SEQ ID NO: 31 - DNA, 23 bp, Artificial Sequence
  Synthetic Polynucleotide
tccagcgaacttcacctgacagg

SEQ ID NO: 32 - DNA, 23 bp, Artificial Sequence
  Synthetic Polynucleotide
ccaagtatccccggactctttgg

SEQ ID NO: 33 - DNA, 23 bp, Artificial Sequence
  Synthetic Polynucleotide
agcattatccaaagagtccgggg

SEQ ID NO: 34 - DNA, 23 bp, Artificial Sequence
  Synthetic Polynucleotide
acttgggtggaagtattgtctgg

SEQ ID NO: 35 - DNA, 23 bp, Artificial Sequence
  Synthetic Polynucleotide
gtctgcgagtctgcgtgcgtggg

SEQ ID NO: 36 - DNA, 23 bp, Artificial Sequence
  Synthetic Polynucleotide
cgtctgcgagtctgcgtgcgtgg

SEQ ID NO: 37 - DNA, 23 bp, Artificial Sequence
  Synthetic Polynucleotide
gcgagtctgcgtgcgtgggaagg

SEQ ID NO: 38 - DNA, 1568 bp, Homo sapiens
  misc_feature (19)..(19): n is a, c, g, or t
ggtgtcgtgagcggccgctgaactggccaccatgtggctgcagtctctgctgctgctgggcaccgtggcctgtagcatcagcgagatcgtgctgacccagagccctggctctctggctgtgtctcctggcgagcgcgtgaccatgagctgcaagagcagccagagcgtgttcttcagcagctcccagaagaactacctggcctggtatcagcagatccccggccagagccccagactgctgatctactgggccagcaccagagaaagcggcgtgcccgatagattcaccggcagcggctctggcaccgacttcaccctgacaatcagcagcgtgcagcccgaggacctggccatctactactgccaccagtacctgagcagccggacctttggccagggcaccaagctggaaatcaagcggggcagcacaagcggcagcggaaagcctggatctggcgagggctctaccaagggccaggtgcagctgcagcagcctggcgccgaagtcgtgaaacctggcgcctccgtgaagatgtcctgcaaggccagcggctacaccttcaccagctactacatccactggatcaagcagacccctggacagggcctggaatgggtgggagtgatctaccccggcaacgacgacatcagctacaaccagaagttccagggcaaggccaccctgaccgccgacaagtctagcaccaccgcctacatgcagctgtccagcctgaccagcgaggacagcgccgtgtactactgcgccagagaagtgcggctgcggtacttcgatgtgtggggccagggaaccaccgtgaccgtgtctagcgccctgagcaacagcatcatgtacttcagccacttcgtgcccgtgtttctgcccgccaagcctaccacaacccctgcccctagacctcctaccccagcccctacaatcgccagccagcctctgtctctgaggcccgaggcttctagaccagctgctggcggagccgtgcacaccagaggcctggatatctacatctgggccccactggccggcacctgtggcgtgctgctgctgtctctcgtgatcaccaagagaggccggaagaagctgctgtacatcttcaagcagcccttcatgcggcccgtgcagaccacccaggaagaggacggctgtagctgccggttccccgaggaagaagaagggggctgcgagctgagagtgaagttcagcagaagcgccgacgcccctgcctatcagcagggccagaaccagctgtacaacgagctgaacctgggcagacgggaagagtacgacgtgctggacaagcggagaggcagggaccctgagatgggcggcaagcccagacggaagaaccctcaggaaggcctgtataacgaactgcagaaagacaagatggccgaggcctactccgagatcggaatgaagggcgagcggagaagaggcaagggccacgatggactgtaccagggcctgagcaccgccaccaaggacacctatgacgccctgcacatgcaggccctgccccccagatgaaattcatcgacgttaactattctag

SEQ ID NO: 39 - DNA, 1586 bp, Homo sapiens
  misc_feature (20)..(20): n is a, c, g, or t
ggtgtcgtgagcggccgctgaactggccaccatgtggctgcagtctctgctgctgctgggcaccgtggcctgtagcatcagcgagatcgtgctgacccagagccctggctctctggctgtgtctcctggcgagcgcgtgaccatgagctgcaagagcagccagagcgtgttcttcagcagctcccagaagaactacctggcctggtatcagcagatccccggccagagccccagactgctgatctactgggccagcaccagagaaagcggcgtgcccgatagattcaccggcagcggctctggcaccgacttcaccctgacaatcagcagcgtgcagcccgaggacctggccatctactactgccaccagtacctgagcagccggacctttggccagggcaccaagctggaaatcaagcggggcagcacaagcggcagcggaaagcctggatctggcgagggctctaccaagggccaggtgcagctgcagcagcctggcgccgaagtcgtgaaacctggcgcctccgtgaagatgtcctgcaaggccagcggctacaccttcaccagctactacatccactggatcaagcagacccctggacagggcctggaatgggtgggagtgatctaccccggcaacgacgacatcagctacaaccagaagttccagggcaaggccaccctgaccgccgacaagtctagcaccaccgcctacatgcagctgtccagcctgaccagcgaggacagcgccgtgtactactgcgccagagaagtgcggctgcggtacttcgatgtgtggggccagggaaccaccgtgaccgtgtctgccctgagcaacagcatcatgtacttcagccacttcgtgcccgtgtttctgcccgccaagcctaccacaacccctgcccctagacctcctaccccagcccctacaatcgccagccagcctctgtctctgaggcccgaggcttctagaccagctgctggcggagccgtgcacaccagaggactggacaagcccttctgggtgctggtggtcgtgggcggagtgctggcctgttacagcctgctcgtgacagtggccttcatcatcttttgggtgcgcagcaagcggtctagactgctgcacagcgactacatgaacatgacccccagaaggccaggccccacccggaagcactatcagccttacgcccctcccagagacttcgccgcctaccggtccagagtgaagttcagcagaagcgccgacgcccctgcctatcagcagggccagaaccagctgtacaacgagctgaacctgggcagacgggaagagtacgacgtgctggacaagagaagaggccgggaccctgagatgggcggcaagcccagacggaagaaccctcaggaaggcctgtataacgaactgcagaaagacaagatggccgaggcctactccgagatcggcatgaagggcgaacggcggagaggcaagggacacgatggactgtaccagggcctgagcaccgccaccaaggacacctatgacgccctgcacatgcaggccctgccccccagatgaaattcatcgacgttaactattctag

SEQ ID NO: 40 - DNA, 1715 bp, Homo sapiens
ggtgtcgtgagcggccgctgaactggccaccatgtggctgcagtctctgctgctgctgggcaccgtggcctgtagcatcagcgagatcgtgctgacccagagccctggctctctggctgtgtctcctggcgagcgcgtgaccatgagctgcaagagcagccagagcgtgttcttcagcagctcccagaagaactacctggcctggtatcagcagatccccggccagagccccagactgctgatctactgggccagcaccagagaaagcggcgtgcccgatagattcaccggcagcggctctggcaccgacttcaccctgacaatcagcagcgtgcagcccgaggacctggccatctactactgccaccagtacctgagcagccggacctttggccagggcaccaagctggaaatcaagcggggcagcacaagcggcagcggaaagcctggatctggcgagggctctaccaagggccaggtgcagctgcagcagcctggcgccgaagtcgtgaaacctggcgcctccgtgaagatgtcctgcaaggccagcggctacaccttcaccagctactacatccactggatcaagcagacccctggacagggcctggaatgggtgggagtgatctaccccggcaacgacgacatcagctacaaccagaagttccagggcaaggccaccctgaccgccgacaagtctagcaccaccgcctacatgcagctgtccagcctgaccagcgaggacagcgccgtgtactactgcgccagagaagtgcggctgcggtacttcgatgtgtggggccagggaaccaccgtgaccgtgtctagcgccctgagcaacagcatcatgtacttcagccacttcgtgcccgtgtttctgcccgccaagcctaccacaacccctgcccctagacctcctaccccagcccctacaatcgccagccagcctctgtctctgaggcccgaggcttctagaccagctgctggcggagccgtgcacaccagaggactggacaagcccttctgggtgctggtggtcgtgggcggagtgctggcctgttacagcctgctcgtgacagtggccttcatcatcttttgggtgcgcagcaagcggtctagactgctgcacagcgactacatgaacatgacccccagaaggccaggccccacccggaagcactatcagccttacgcccctcccagagacttcgccgcctacagatccaagagaggccggaagaagctgctgtacatcttcaagcagcccttcatgcggcccgtgcagaccacccaggaagaggacggctgtagctgccggttccccgaggaagaagaagggggctgcgagctgagagtgaagttcagcagaagcgccgacgcccctgcctatcagcagggccagaaccagctgtacaacgagctgaacctgggcagacgggaagagtacgacgtgctggacaagagaagaggccgggaccctgagatgggcggcaagcccagacggaagaaccctcaggaaggcctgtataacgaactgcagaaagacaagatggccgaggcctactccgagatcggaatgaagggcgagcggcggagaggcaagggacacgatggactgtaccagggcctgagcaccgccaccaaggacacctatgacgccctgcacatgcaggccctgccccccagatgaaattcatcgacgttaactattctag

SEQ ID NO: 41 - DNA, 1436 bp, Homo sapiens
ggtgtcgtgagcggccgctgaactggccaccatgtggctgcagtctctgctgctgctgggcaccgtggcctgcagcatcagcatccagatgacccagaccaccagcagcctgagcgccagcctgggcgatagagtgaccatcagctgcagagccagccaggacatcagcaagtacctgaactggtatcagcagaaacccgacggcaccgtgaagctgctgatctaccacaccagcagactgcacagcggcgtgccctctagattttccggcagcggctccggcaccgactacagcctgaccatctccaacctggaacaggaagatatcgctacctacttctgtcagcaaggcaacaccctgccctacaccttcggcggaggcaccaagctggaaatcggcagcacaagcggctctggcaagcctggatctggcgagggctctaccaagggcctgcaggaatctggccctggactggtggcccctagccagagcctgtctgtgacctgtaccgtgtccggcgtgtccctgcctgactatggcgtgtcctggatcagacagccccccagaaagggcctggaatggctgggagtgatctggggcagcgagacaacctactacaacagcgccctgaagtcccggctgaccatcatcaaggacaactccaagagccaggtgttcctgaagatgaacagcctgcagaccgacgacaccgccatctactactgcgccaagcactactactacggcggcagctacgccatggactactggggccagggcacaagcgtgaccgtgtctgccctgagcaacagcatcatgtacttcagccacttcgtgcccgtgtttctgcccgccaagcctaccacaacccctgcccctagacctcctaccccagcccctacaatcgccagccagcctctgtctctgaggcccgaggcttctagaccagctgctggcggagccgtgcacaccagaggactggacaagcccttctgggtgctggtggtcgtgggcggagtgctggcctgttatagcctgctcgtgacagtggccttcatcatcttttgggtgcgcgtgaagttcagccgcagcgccgatgcccctgcctatcagcagggacagaaccagctgtacaacgagctgaacctgggcagacgggaagagtacgacgtgctggacaagagaagaggccgggaccctgagatgggcggcaagcccagaagaaagaacccccaggaaggcctgtataacgaactgcagaaagacaagatggccgaggcctacagcgagatcggcatgaagggcgaacggcggagaggcaagggccacgatggactgtatcagggcctgagcaccgccaccaaggacacctatgacgccctgcacatgcaggctctgccccctcgctgaaattcatcgacgttaactattctag

SEQ ID NO: 42 - DNA, 1253 bp, Homo sapiens
ggtgtcgtgagcggccgctgaactggccaccatgtggctgcagtctctgctgctgctgggcaccgtggcctgtagcatcagcgagatcgtgctgacccagagccctggctctctggctgtgtctcctggcgagcgcgtgaccatgagctgcaagagcagccagagcgtgttcttcagcagctcccagaagaactacctggcctggtatcagcagatccccggccagagccccagactgctgatctactgggccagcaccagagaaagcggcgtgcccgatagattcaccggcagcggctctggcaccgacttcaccctgacaatcagcagcgtgcagcccgaggacctggccatctactactgccaccagtacctgagcagccggacctttggccagggcaccaagctggaaatcaagcggggcagcacaagcggcagcggaaagcctggatctggcgagggctctaccaagggccaggtgcagctgcagcagcctggcgccgaagtcgtgaaacctggcgcctccgtgaagatgtcctgcaaggccagcggctacaccttcaccagctactacatccactggatcaagcagacccctggacagggcctggaatgggtgggagtgatctaccccggcaacgacgacatcagctacaaccagaagttccagggcaaggccaccctgaccgccgacaagtctagcaccaccgcctacatgcagctgtccagcctgaccagcgaggacagcgccgtgtactactgcgccagagaagtgcggctgcggtacttcgatgtgtggggccagggaaccaccgtgaccgtgtctagcgccctgagcaacagcatcatgtacttcagccacttcgtgcccgtgtttctgcccgccaagcctaccacaacccctgcccctagacctcctaccccagcccctacaatcgccagccagcctctgtctctgaggcccgaggcttctagaccagctgctggcggagccgtgcacaccagaggactggacaagcccttctgggtgctggtggtcgtgggcggagtgctggcctgttacagcctgctcgtgacagtggccttcatcatcttttgggtgcgcagcaagcggtctagactgctgcacagcgactacatgaacatgacccccagaaggccaggccccacccggaagcactatcagccttacgcccctcccagagacttcgccgcctacagaagctgaaattcatcgacgttaactattctag

SEQ ID NO: 43 - DNA, 1559 bp, Homo sapiens
ggtgtcgtgagcggccgctgaactggccaccatgtggctgcagtctctgctgctgctgggcaccgtggcctgcagcatcagcatccagatgacccagaccaccagcagcctgagcgccagcctgggcgatagagtgaccatcagctgcagagccagccaggacatcagcaagtacctgaactggtatcagcagaaacccgacggcaccgtgaagctgctgatctaccacaccagcagactgcacagcggcgtgccctctagattttccggcagcggctccggcaccgactacagcctgaccatctccaacctggaacaggaagatatcgctacctacttctgtcagcaaggcaacaccctgccctacaccttcggcggaggcaccaagctggaaatcggcagcacaagcggctctggcaagcctggatctggcgagggctctaccaagggcctgcaggaatctggccctggactggtggcccctagccagagcctgtctgtgacctgtaccgtgtccggcgtgtccctgcctgactatggcgtgtcctggatcagacagccccccagaaagggcctggaatggctgggagtgatctggggcagcgagacaacctactacaacagcgccctgaagtcccggctgaccatcatcaaggacaactccaagagccaggtgttcctgaagatgaacagcctgcagaccgacgacaccgccatctactactgcgccaagcactactactacggcggcagctacgccatggactactggggccagggcacaagcgtgaccgtgtctgccctgagcaacagcatcatgtacttcagccacttcgtgcccgtgtttctgcccgccaagcctaccacaacccctgcccctagacctcctaccccagcccctacaatcgccagccagcctctgtctctgaggcccgaggcttctagaccagctgctggcggagccgtgcacaccagaggactggacaagcccttctgggtgctggtggtcgtgggcggagtgctggcctgttatagcctgctcgtgacagtggccttcatcatcttttgggtgcgcagcaagcggagccggctgctgcactccgactacatgaacatgacccccagacggccaggccccacccggaaacactatcagccttacgcccctcccagagacttcgccgcctaccggtccagagtgaagttcagcagatccgccgacgcccctgcctatcagcagggacagaaccagctgtacaacgagctgaacctgggcagacgggaagagtacgacgtgctggacaagagaagaggccgggaccctgagatgggcggcaagcccagaagaaagaacccccaggaaggcctgtataacgaactgcagaaagacaagatggccgaggcctacagcgagatcggcatgaagggcgaacggcggagaggcaagggccacgatggactgtatcagggcctgagcaccgccaccaaggacacctatgacgccctgcacatgcaggctctgccccctcgctgaaattcatcgacgttaactattctag

SEQ ID NO: 44 - DNA, 1514 bp, Homo sapiens
ggtgtcgtgagcggccgctgaactggccaccatgtggctgcagtctctgctgctgctgggcaccgtggcctgtagcatcagcgagatcgtgctgacccagagccctggctctctggctgtgtctcctggcgagcgcgtgaccatgagctgcaagagcagccagagcgtgttcttcagcagctcccagaagaactacctggcctggtatcagcagatccccggccagagccccagactgctgatctactgggccagcaccagagaaagcggcgtgcccgatagattcaccggcagcggctctggcaccgacttcaccctgacaatcagcagcgtgcagcccgaggacctggccatctactactgccaccagtacctgagcagccggacctttggccagggcaccaagctggaaatcaagcggggcagcacaagcggcagcggaaagcctggatctggcgagggctctaccaagggccaggtgcagctgcagcagcctggcgccgaagtcgtgaaacctggcgcctccgtgaagatgtcctgcaaggccagcggctacaccttcaccagctactacatccactggatcaagcagacccctggacagggcctggaatgggtgggagtgatctaccccggcaacgacgacatcagctacaaccagaagttccagggcaaggccaccctgaccgccgacaagtctagcaccaccgcctacatgcagctgtccagcctgaccagcgaggacagcgccgtgtactactgcgccagagaagtgcggctgcggtacttcgatgtgtggggccagggaaccaccgtgaccgtgtccagcatcgaagtgatgtacccccctccctacctggacaacgagaagtccaacggcaccatcatccacgtgaagggcaagcacctgtgccccagccctctgtttcctggccctagcaagcccttctgggtgctggtggtcgtgggcggagtgctggcctgttacagcctgctcgtgacagtggccttcatcatcttttgggtgcgcagcaagcggtctagactgctgcacagcgactacatgaacatgacccccagaaggccaggccccacccggaagcactatcagccttacgcccctcccagagacttcgccgcctaccggtccagagtgaagttcagcagaagcgccgacgcccctgcctatcagcagggccagaaccagctgtacaacgagctgaacctgggcagacgggaagagtacgacgtgctggacaagcggagaggcagggaccctgagatgggcggcaagcccagacggaagaaccctcaggaaggcctgtataacgaactgcagaaagacaagatggccgaggcctactccgagatcggcatgaagggcgagcggagaagaggcaagggccacgatggactgtaccagggcctgagcaccgccaccaaggacacctatgacgccctgcacatgcaggccctgccccccagatgaaattcatcgacgttaactattctag

SEQ ID NO: 45 - DNA, 21 bp, Artificial Sequence
  Synthetic Polynucleotide
  misc_feature (19)..(19): n is a, c, g, or t
atcgatcgatcgtacgcgngg

SEQ ID NO: 46 - DNA, 22 bp, Artificial Sequence
  Synthetic Polynucleotide
  misc_feature (20)..(20): n is a, c, g, or t
atgcatcgtacatcgatcgngg

SEQ ID NO: 47 - protein, 38 aa, Artificial Sequence
  Synthetic Polypeptide
CWLTKKKYSSSVHDPNGEYMFMRAVNTAKKSRLTDVTL